European Patent Application EP 4 282 873 A1, published November 29, 2023. Title: Method for screening dimerized cyclic peptide. Applicant: Ajinomoto Co., Inc. The sequence listing filed with the application follows.

SEQUENCE LISTING (90 sequences)

SEQ ID NO: 1 - protein, 17 aa, Artificial Sequence
  Met binding peptide
  DISULFID (1)..(17): Disulfide bridge between Cys-1 and Cys-17
CYRQFNRRTHEVWNLDC

SEQ ID NO: 2 - protein, 16 aa, Artificial Sequence
  Met binding peptide
  DISULFID (1)..(16): Disulfide bridge between Cys-1 and Cys-16
CRQFNRRTHEVWNLDC

SEQ ID NO: 3 - protein, 16 aa, Artificial Sequence
  Met binding peptide
  DISULFID (1)..(16): Disulfide bridge between Cys-1 and Cys-16
CYWYYAWDQTYKAFPC

SEQ ID NO: 4 - protein, 15 aa, Artificial Sequence
  Met binding peptide
  DISULFID (1)..(15): Disulfide bridge between Cys-1 and Cys-15
CWYYAWDQTYKAFPC

SEQ ID NO: 5 - protein, 18 aa, Artificial Sequence
  Met binding peptide
  DISULFID (1)..(18): Disulfide bridge between Cys-1 and Cys-18
CYISWNEFNSPNWRFITC

SEQ ID NO: 6 - protein, 17 aa, Artificial Sequence
  Met binding peptide
  DISULFID (1)..(17): Disulfide bridge between Cys-1 and Cys-17
CISWNEFNSPNWRFITC

SEQ ID NO: 7 - protein, 20 aa, Artificial Sequence
  EpoR binding peptide
  DISULFID (6)..(15): Disulfide bridge between Cys-6 and Cys-15
GGLYACHMGPMTWVCQPLRG

SEQ ID NO: 8 - protein, 17 aa, Artificial Sequence
  EpoR binding peptide
  DISULFID (1)..(17): Disulfide bridge between Cys-1 and Cys-17
CISWNEFNSPNWRFITC

SEQ ID NO: 9 - protein, 20 aa, Artificial Sequence
  PAS Linker
AAPAAPAPAAPAAPAPAAPA

SEQ ID NO: 10 - protein, 22 aa, Artificial Sequence
  PAS Linker
AAPAAPAPAAPAAPAPAAPAAP

SEQ ID NO: 11 - protein, 14 aa, Artificial Sequence
  PAS Linker
AAPAAPAPAAPAAP

SEQ ID NO: 12 - protein, 20 aa, Artificial Sequence
  PAS Linker
AAPAAAPAPAAPAAPAPAAP

SEQ ID NO: 13 - protein, 20 aa, Artificial Sequence
  PAS Linker
AAAPAAAPAAAPAAAPAAAP

SEQ ID NO: 14 - protein, 24 aa, Artificial Sequence
  PAS Linker
AAPAAPAAPAAPAAPAAPAAPAAP

SEQ ID NO: 15 - protein, 24 aa, Artificial Sequence
  PAS Linker
APAAAPAPAAAPAPAAAPAPAAAP

SEQ ID NO: 16 - protein, 24 aa, Artificial Sequence
  PAS Linker
AAAPAAPAAPPAAAAPAAPAAPPA

SEQ ID NO: 17 - protein, 20 aa, Artificial Sequence
  PAS Linker
APAPAPAPAPAPAPAPAPAP

SEQ ID NO: 18 - protein, 20 aa, Artificial Sequence
  PAS Linker
ASPAAPAPASPAAPAPSAPA

SEQ ID NO: 19 - protein, 20 aa, Artificial Sequence
  PAS Linker
AAPASPAPAAPSAPAPAAPS

SEQ ID NO: 20 - protein, 20 aa, Artificial Sequence
  PAS Linker
APSSPSPSAPSSPSPASPSS

SEQ ID NO: 21 - protein, 20 aa, Artificial Sequence
  PAS Linker
SAPSSPSPSAPSSPSPASPS

SEQ ID NO: 22 - protein, 20 aa, Artificial Sequence
  PAS Linker
SSPSAPSPSSPASPSPSSPA

SEQ ID NO: 23 - protein, 24 aa, Artificial Sequence
  PAS Linker
AASPAAPSAPPAAASPAAPSAPPA

SEQ ID NO: 24 - protein, 20 aa, Artificial Sequence
  PAS Linker
ASAAAPAAASAAASAPSAAA

SEQ ID NO: 25 - protein, 16 aa, Artificial Sequence
  PAS Linker
AAPAAPAPAAPAAPAP

SEQ ID NO: 26 - protein, 49 aa, Artificial Sequence
  PAS Linker
AAPAAPAPAAPAAPAPAAPAAPAPAAPAAPAPAAPAAPAPAAPAAPAPA

SEQ ID NO: 27 - protein, 49 aa, Artificial Sequence
  PAS Linker
SAPSPSSAPASASAPASPASASASASPASSPASASSASPAASSASPASS

SEQ ID NO: 28 - protein, 20 aa, Artificial Sequence
  PAS Linker
APAAPAPAAPAAPAPAAPAA

SEQ ID NO: 29 - protein, 20 aa, Artificial Sequence
  PAS Linker
PAAPAPAAPAAPAPAAPAAA

SEQ ID NO: 30 - protein, 20 aa, Artificial Sequence
  PAS Linker
AAPAPAAPAAPAPAAPAAAP

SEQ ID NO: 31 - protein, 20 aa, Artificial Sequence
  PAS Linker
APAPAAPAAPAPAAPAAAPA

SEQ ID NO: 32 - protein, 20 aa, Artificial Sequence
  PAS Linker
PAPAAPAAPAPAAPAAAPAA

SEQ ID NO: 33 - protein, 20 aa, Artificial Sequence
  PAS Linker
APAAPAAPAPAAPAAAPAAP

SEQ ID NO: 34 - protein, 20 aa, Artificial Sequence
  PAS Linker
PAAPAAPAPAAPAAAPAAPA

SEQ ID NO: 35 - protein, 20 aa, Artificial Sequence
  PAS Linker
AAPAAPAPAAPAAAPAAPAP

SEQ ID NO: 36 - protein, 20 aa, Artificial Sequence
  PAS Linker
APAAPAPAAPAAAPAAPAPA

SEQ ID NO: 37 - protein, 20 aa, Artificial Sequence
  PAS Linker
PAAPAPAAPAAAPAAPAPAA

SEQ ID NO: 38 - protein, 10 aa, Artificial Sequence
  PAS Linker
AAPAAPAPAA

SEQ ID NO: 39 - protein, 8 aa, Artificial Sequence
  PAS Linker
AAPAAPAP

SEQ ID NO: 40 - protein, 9 aa, Artificial Sequence
  PAS Linker
AAPAAPAPA

SEQ ID NO: 41 - protein, 39 aa, Artificial Sequence
  Leucine zipper domain of c-Jun
RIARLEEKVKTLKAQNSELASTANMLREQVAQLKQKVMN

SEQ ID NO: 42 - protein, 39 aa, Artificial Sequence
  Leucine zipper domain of Jun ¢hep
QIAQLEEKVQTLQAQNSELASTANMLREQVAQLKQKVMN

SEQ ID NO: 43 - protein, 33 aa, Artificial Sequence
  Leucine zipper domain of GCN4
RMKQLEDKVEELLSKNYHLENEVARLKKLVGER

SEQ ID NO: 44 - protein, 39 aa, Artificial Sequence
  Leucine zipper domain of CEBP ¿
RNVETQQKVLELTSDNDRLRKRVEQLSRELDTLRGIFRQ

SEQ ID NO: 45 - protein, 74 aa, Artificial Sequence
  aMD4dY-PA8-cys-Jun
  DISULFID (5)..(20): Disulfide bridge between Cys-5 and Cys-20
MAETCRQFNRRTHEVWNLDCGAAPAAPAPAAGCGGRIARLEEKVKTLKAQNSELASTANMLREQVAQLKQKVMN

SEQ ID NO: 46 - protein, 73 aa, Artificial Sequence
  aMD4dY-PA8-Jun
  DISULFID (5)..(20): Disulfide bridge between Cys-5 and Cys-20
MAETCRQFNRRTHEVWNLDCGAAPAAPAPAAGGGRIARLEEKVKTLKAQNSELASTANMLREQVAQLKQKVMN

SEQ ID NO: 47 - protein, 74 aa, Artificial Sequence
  aMD4dY-PA8-cys-Jun ¢hep
  DISULFID (5)..(20): Disulfide bridge between Cys-5 and Cys-20
MAETCRQFNRRTHEVWNLDCGAAPAAPAPAAGCGGQIAQLEEKVQTLQAQNSELASTANMLREQVAQLKQKVMN

SEQ ID NO: 48 - protein, 68 aa, Artificial Sequence
  aMD4dY-PA8-GCN4-cys
  DISULFID (5)..(20): Disulfide bridge between Cys-5 and Cys-20
MAETCRQFNRRTHEVWNLDCGAAPAAPAPGRMKQLEDKVEELLSKNYHLENEVARLKKLVGERGGCGG

SEQ ID NO: 49 - protein, 74 aa, Artificial Sequence
  aMD4dY-PA8-cys-CEBP ¿
  DISULFID (5)..(20): Disulfide bridge between Cys-5 and Cys-20
MAETCRQFNRRTHEVWNLDCGAAPAAPAPAAGCGGRNVETQQKVLELTSDNDRLRKRVEQLSRELDTLRGIFRQ

SEQ ID NO: 50 - protein, 70 aa, Artificial Sequence
  cys-Jun-PA8-aMD4dY
  DISULFID (55)..(70): Disulfide bridge between Cys-55 and Cys-70
MGGCGGRIARLEEKVKTLKAQNSELASTANMLREQVAQLKQKVMNAAPAAPAPACRQFNRRTHEVWNLDC

SEQ ID NO: 51 - protein, 71 aa, Artificial Sequence
  Jun-cys-PA8-aMD4dY
  DISULFID (56)..(71): Disulfide bridge between Cys-56 and Cys-71
MGRIARLEEKVKTLKAQNSELASTANMLREQVAQLKQKVMNGGCGGAAPAAPAPACRQFNRRTHEVWNLDC

SEQ ID NO: 52 - protein, 91 aa, Artificial Sequence
  N11-Jun-cys-PA8-aMD4dY
  DISULFID (76)..(91): Disulfide bridge between Cys-76 and Cys-91
MKDHLIHNHHKHEHAHAEHLGGRIARLEEKVKTLKAQNSELASTANMLREQVAQLKQKVMNGGCGGAAPAAPAPACRQFNRRTHEVWNLDC

SEQ ID NO: 53 - protein, 89 aa, Artificial Sequence
  N11-cys-Jun-PA8-aMD4dY
  DISULFID (74)..(89): Disulfide bridge between Cys-74 and Cys-89
MKDHLIHNHHKHEHAHAEHLGGCGGRIARLEEKVKTLKAQNSELASTANMLREQVAQLKQKVMNAAPAAPAPACRQFNRRTHEVWNLDC

SEQ ID NO: 54 - protein, 85 aa, Artificial Sequence
  N11-GCN4-cys-PA8-aMD4dY
  DISULFID (70)..(85): Disulfide bridge between Cys-70 and Cys-85
MKDHLIHNHHKHEHAHAEHLGGRMKQLEDKVEELLSKNYHLENEVARLKKLVGERGGCGGAAPAAPAPACRQFNRRTHEVWNLDC

SEQ ID NO: 55 - protein, 83 aa, Artificial Sequence
  N11-cys-GCN4-PA8-aMD4dY
  DISULFID (68)..(83): Disulfide bridge between Cys-68 and Cys-83
MKDHLIHNHHKHEHAHAEHLGGCGGRMKQLEDKVEELLSKNYHLENEVARLKKLVGERAAPAAPAPACRQFNRRTHEVWNLDC

SEQ ID NO: 56 - DNA, 324 bp, Artificial Sequence
  aMD4dY-PA8-cys-Jun
gaaattaatacgactcactatagggagaccacaacggtttccctctagaaataattttgtttaactttaagaaggagatataccaatggcagagacctgtcgtcagtttaaccgtcgtacgcacgaagtttggaatctggactgtggcgcagcccccgcagcaccagctccagcagcaggctgcggtggtcgtatcgctcgtctggaagaaaaagttaaaaccctgaaagctcagaactccgaactggcttccaccgctaacatgctgcgtgaacaggttgctcagctgaaacagaaagttatgaactagtgaataactaatcc

SEQ ID NO: 57 - DNA, 321 bp, Artificial Sequence
  aMD4dY-PA8-Jun
gaaattaatacgactcactatagggagaccacaacggtttccctctagaaataattttgtttaactttaagaaggagatataccaatggcagagacctgtcgtcagtttaaccgtcgtacgcacgaagtttggaatctggactgtggcgcagcccccgcagcaccagctccagcagcaggcggtggtcgtatcgctcgtctggaagaaaaagttaaaaccctgaaagctcagaactccgaactggcttccaccgctaacatgctgcgtgaacaggttgctcagctgaaacagaaagttatgaactagtgaataactaatcc

SEQ ID NO: 58 - DNA, 324 bp, Artificial Sequence
  aMD4dY-PA8-cys-Jun ¢hep
gaaattaatacgactcactatagggagaccacaacggtttccctctagaaataattttgtttaactttaagaaggagatataccaatggcagagacctgtcgtcagtttaaccgtcgtacgcacgaagtttggaatctggactgtggcgcagcccccgcagcaccagctccagcagcaggctgcggtggtcagattgcccaactggaagagaaagtgcagacgttacaagcgcaaaacagcgaactggcttcgaccgcgaacatgttgcgcgaacaggttgcacagctgaaacagaaggtcatgaattagtgaataactaatcc

SEQ ID NO: 59 - DNA, 306 bp, Artificial Sequence
  aMD4dY-PA8-GCN4-cys
gaaattaatacgactcactatagggagaccacaacggtttccctctagaaataattttgtttaactttaagaaggagatataccaatggcagagacctgtcgtcagtttaaccgtcgtacgcacgaagtttggaatctggactgtggcgcagcacccgcagctccagcaccaggccgcatgaaacagttggaggataaagtcgaagagcttctgagcaagaactatcacctcgaaaacgaagttgctcgtctgaagaaactcgttggagaacgtggtggttgtggcgggtagtgaataactaatcc

SEQ ID NO: 60 - DNA, 324 bp, Artificial Sequence
  aMD4dY-PA8-cys-CEBP ¿
gaaattaatacgactcactatagggagaccacaacggtttccctctagaaataattttgtttaactttaagaaggagatataccaatggcagagacctgtcgtcagtttaaccgtcgtacgcacgaagtttggaatctggactgtggcgcagcccccgcagcaccagctccagcagcaggctgcggtggtcgcaatgtggagactcagcagaaggtcctggaactgacgtctgacaacgatcggttacgcaaacgggttgaacagctgtctcgtgaactcgacactcttcgtggcatcttccgccaatagtgaataactaatcc

SEQ ID NO: 61 - DNA, 312 bp, Artificial Sequence
  cys-Jun-PA8-aMD4dY
gaaattaatacgactcactatagggagaccacaacggtttccctctagaaataattttgtttaactttaagaaggagatataccaatgggtggttgcggtggtcgtatcgctcgtctggaagaaaaagttaaaaccctgaaagctcagaactccgaactggcttccaccgctaacatgctgcgtgaacaggttgctcagctgaaacagaaagttatgaacgcagcccccgcagcaccagctccagcatgtcgtcagtttaaccgtcgtacgcacgaagtttggaatctggactgttagtgaataactaatcc

SEQ ID NO: 62 - DNA, 315 bp, Artificial Sequence
  Jun-cys-PA8-aMD4dY
gaaattaatacgactcactatagggagaccacaacggtttccctctagaaataattttgtttaactttaagaaggagatataccaatgggtcgtatcgctcgtctggaagaaaaagttaaaaccctgaaagctcagaactccgaactggcttccaccgctaacatgctgcgtgaacaggttgctcagctgaaacagaaagttatgaacggtggttgcggtggtgcagcccccgcagcaccagctccagcatgtcgtcagtttaaccgtcgtacgcacgaagtttggaatctggactgttagtgaataactaatcc

SEQ ID NO: 63 - DNA, 375 bp, Artificial Sequence
  N11-Jun-cys-PA8-aMD4dY
gaaattaatacgactcactatagggagaccacaacggtttccctctagaaataattttgtttaactttaagaaggagatataccaatgaaagatcatctcatccacaatcatcacaaacatgagcacgctcatgccgaacacctgggtggtcgtatcgctcgtctggaagaaaaagttaaaaccctgaaagctcagaactccgaactggcttccaccgctaacatgctgcgtgaacaggttgctcagctgaaacagaaagttatgaacggtggttgcggtggtgcagcaccagcagctccggcccctgcttgtcgtcagtttaaccgtcgtacgcacgaagtttggaatctggactgttagtgaataactaatcc

SEQ ID NO: 64 - DNA, 369 bp, Artificial Sequence
  N11-GCN4-cys-PA8-aMD4dY
gaaattaatacgactcactatagggagaccacaacggtttccctctagaaataattttgtttaactttaagaaggagatataccaatgaaagatcatctcatccacaatcatcacaaacatgagcacgctcatgccgaacacctgggtggttgcggtggtcgtatcgctcgtctggaagaaaaagttaaaaccctgaaagctcagaactccgaactggcttccaccgctaacatgctgcgtgaacaggttgctcagctgaaacagaaagttatgaacgcagcaccagcagctccggcccctgcttgtcgtcagtttaaccgtcgtacgcacgaagtttggaatctggactgttagtgaataactaatcc

SEQ ID NO: 65 - DNA, 357 bp, Artificial Sequence
  N11-GCN4-cys-PA8-aMD4dY
gaaattaatacgactcactatagggagaccacaacggtttccctctagaaataattttgtttaactttaagaaggagatataccaatgaaagatcatctcatccacaatcatcacaaacatgagcacgctcatgccgaacacctgggtggtcgcatgaaacagttggaggataaagtcgaagagcttctgagcaagaactatcacctcgaaaacgaagttgctcgtctgaagaaactcgttggagaacgtggtggttgcggtggtgcagcaccagcagctccggcccctgcttgtcgtcagtttaaccgtcgtacgcacgaagtttggaatctggactgttagtgaataactaatcc

SEQ ID NO: 66 - DNA, 351 bp, Artificial Sequence
  N11-cys-GCN4-PA8-aMD4dY
gaaattaatacgactcactatagggagaccacaacggtttccctctagaaataattttgtttaactttaagaaggagatataccaatgaaagatcatctcatccacaatcatcacaaacatgagcacgctcatgccgaacacctgggtggttgcggtggtcgcatgaaacagttggaggataaagtcgaagagcttctgagcaagaactatcacctcgaaaacgaagttgctcgtctgaagaaactcgttggagaacgtgcagcaccagcagctccggcccctgcttgtcgtcagtttaaccgtcgtacgcacgaagtttggaatctggactgttagtgaataactaatcc

SEQ ID NO: 67 - protein, 74 aa, Artificial Sequence
  EMP-PA8-cys-Jun
  DISULFID (7)..(16): Disulfide bridge between Cys-7 and Cys-16
MGGLYACHMGPMTWVCQPLRGAAPAAPAPAAGCGGRIARLEEKVKTLKAQNSELASTANMLREQVAQLKQKVMN

SEQ ID NO: 68 - DNA, 324 bp, Artificial Sequence
  EMP-PA8-cys-Jun
gaaattaatacgactcactatagggagaccacaacggtttccctctagaaataattttgtttaactttaagaaggagatataccaatgggtggcctgtatgcgtgccatatggggccaatgacctgggtgtgtcagccgttacgcggcgcagcccccgcagcaccagctccagcagcaggctgcggtggtcgtatcgctcgtctggaagaaaaagttaaaaccctgaaagctcagaactccgaactggcttccaccgctaacatgctgcgtgaacaggttgctcagctgaaacagaaagttatgaactagtgaataactaatcc

SEQ ID NO: 69 - DNA, 25 bp, Artificial Sequence
  Cell-free primer Fwd
gaaattaatacgactcactataggg

SEQ ID NO: 70 - DNA, 23 bp, Artificial Sequence
  Cell-free primer Rev
cactgactggattagttattcac

SEQ ID NO: 71 - protein, 117 aa, Artificial Sequence
  aMD4dY-Jun-cys-N11-SecM-GS3
  DISULFID (5)..(20): Disulfide bridge between Cys-5 and Cys-20
MAETCRQFNRRTHEVWNLDCGAAPAAPAPAAGGRIARLEEKVKTLKAQNSELASTANMLREQVAQLKQKVMNGCGGKDHLIHNHHKHEHAHAEHLFSTPVWISQAQGIRAGGSGSGS

SEQ ID NO: 72 - protein, 115 aa, Artificial Sequence
  TPO-Jun-cys-N11-SecM-GS3
  DISULFID (5)..(18): Disulfide bridge between Cys-5 and Cys-18
MAETCADGPTLREWISFCGAAPAAPAPAAGGRIARLEEKVKTLKAQNSELASTANMLREQVAQLKQKVMNGCGGKDHLIHNHHKHEHAHAEHLFSTPVWISQAQGIRAGGSGSGS

SEQ ID NO: 73 - protein, 111 aa, Artificial Sequence
  EMP'-Jun-cys-N11-SecM-GS3
  DISULFID (5)..(14): Disulfide bridge between Cys-5 and Cys-14
MAETCHMGPMTWVCGAAPAAPAPAAGGRIARLEEKVKTLKAQNSELASTANMLREQVAQLKQKVMNGCGGKDHLIHNHHKHEHAHAEHLFSTPVWISQAQGIRAGGSGSGS

SEQ ID NO: 74 - DNA, 453 bp, Artificial Sequence
  aMD4dY-Jun-cys-N11-SecM-GS3
gaaattaatacgactcactatagggagaccacaacggtttccctctagaaataattttgtttaactttaagaaggagatataccaatggcagagacctgtcgtcagtttaaccgtcgtacgcacgaagtttggaatctggactgtggcgcagctcccgcagcaccagctccagcagcaggcggtcgtatcgctcgtctggaagaaaaagttaaaaccctgaaagctcagaactccgaactggcttccaccgctaacatgctgcgtgaacaggttgctcagctgaaacagaaagttatgaacggctgcggtggcaaagatcatctcatccacaatcatcacaaacatgagcacgctcatgccgaacacctgttttctactcctgtttggatttctcaagctcaaggtattcgtgctggtggtagcggtagcggtagctagtgaataactaatcc

SEQ ID NO: 75 - DNA, 447 bp, Artificial Sequence
  TPO-Jun-cys-N11-SecM-GS3
gaaattaatacgactcactatagggagaccacaacggtttccctctagaaataattttgtttaactttaagaaggagatataccaatggcagagacctgtgcggacggtccgacgttacgcgaatggatcagcttttgtggcgcagctcccgcagcaccagctccagcagcaggcggtcgtatcgctcgtctggaagaaaaagttaaaaccctgaaagctcagaactccgaactggcttccaccgctaacatgctgcgtgaacaggttgctcagctgaaacagaaagttatgaacggctgcggtggcaaagatcatctcatccacaatcatcacaaacatgagcacgctcatgccgaacacctgttttctactcctgtttggatttctcaagctcaaggtattcgtgctggtggtagcggtagcggtagctagtgaataactaatcc

SEQ ID NO: 76 - DNA, 435 bp, Artificial Sequence
  EMP'-Jun-cys-N11-SecM-GS3
gaaattaatacgactcactatagggagaccacaacggtttccctctagaaataattttgtttaactttaagaaggagatataccaatggcagagacctgtcatatggggccaatgacctgggtgtgtggcgcagctcccgcagcaccagctccagcagcaggcggtcgtatcgctcgtctggaagaaaaagttaaaaccctgaaagctcagaactccgaactggcttccaccgctaacatgctgcgtgaacaggttgctcagctgaaacagaaagttatgaacggctgcggtggcaaagatcatctcatccacaatcatcacaaacatgagcacgctcatgccgaacacctgttttctactcctgtttggatttctcaagctcaaggtattcgtgctggtggtagcggtagcggtagctagtgaataactaatcc

SEQ ID NO: 77 - DNA, 76 bp, Artificial Sequence
  ssDNA1
caatggcagagacctgtcgtcagtttaaccgtcgtacgcacgaagtttggaatctggactgtggcgcagctcccgc

SEQ ID NO: 78 - DNA, 70 bp, Artificial Sequence
  ssDNA2
caatggcagagacctgtgcggacggtccgacgttacgcgaatggatcagcttttgtggcgcagctcccgc

SEQ ID NO: 79 - DNA, 58 bp, Artificial Sequence
  ssDNA3
caatggcagagacctgtcatatggggccaatgacctgggtgtgtggcgcagctcccgc

SEQ ID NO: 80 - DNA, 100 bp, Artificial Sequence
  ssDNA4
gaaattaatacgactcactatagggagaccacaacggtttccctctagaaataattttgtttaactttaagaaggagatataccaatggcagagacctgt

SEQ ID NO: 81 - DNA, 159 bp, Artificial Sequence
  ssDNA5
tgtggcgcagctcccgcagcaccagctccagcagcaggcggtcgtatcgctcgtctggaagaaaaagttaaaaccctgaaagctcagaactccgaactggcttccaccgctaacatgctgcgtgaacaggttgctcagctgaaacagaaagttatgaac

SEQ ID NO: 82 - DNA, 139 bp, Artificial Sequence
  ssDNA6
accagcacgaataccttgagcttgagaaatccaaacaggagtagaaaacaggtgttcggcatgagcgtgctcatgtttgtgatgattgtggatgagatgatctttgccaccgcagccgttcataactttctgtttcagc

SEQ ID NO: 83 - DNA, 53 bp, Artificial Sequence
  ssDNA7
ggattagttattcactagctaccgctaccgctaccaccagcacgaataccttg

SEQ ID NO: 84 - DNA, 39 bp, Artificial Sequence
  ssDNA (selec_PCR_F1.F39)
gaaattaatacgactcactatagggagaccacaacggtt

SEQ ID NO: 85 - DNA, 24 bp, Artificial Sequence
  ssDNA (selec_PCR_R2.R24)
ggattagttattcactagctaccg

SEQ ID NO: 86 - protein, 16 aa, Artificial Sequence
  SecM sequence
FSTPVWISQAQGIRAG

SEQ ID NO: 87 - protein, 120 aa, Artificial Sequence
  EMP-Jun-cys-N11-SecM-GS3
  DISULFID (10)..(19): Disulfide bridge between Cys-10 and Cys-19
MAETGGLYACHMGPMTWVCQPLRGAAPAAPAPAAGGRIARLEEKVKTLKAQNSELASTANMLREQVAQLKQKVMNGCGGKDHLIHNHHKHEHAHAEHLFSTPVWISQAQGIRAGGSGSGS

SEQ ID NO: 88 - DNA, 462 bp, Artificial Sequence
  EMP-Jun-cys-N11-SecM-GS3
gaaattaatacgactcactatagggagaccacaacggtttccctctagaaataattttgtttaactttaagaaggagatataccaatggcagagaccggtggcctgtatgcgtgccatatggggccaatgacctgggtgtgtcagccgttacgcggcgcagctcccgcagcaccagctccagcagcaggcggtcgtatcgctcgtctggaagaaaaagttaaaaccctgaaagctcagaactccgaactggcttccaccgctaacatgctgcgtgaacaggttgctcagctgaaacagaaagttatgaacggctgcggtggcaaagatcatctcatccacaatcatcacaaacatgagcacgctcatgccgaacacctgttttctactcctgtttggatttctcaagctcaaggtattcgtgctggtggtagcggtagcggtagctagtgaataactaatcc

SEQ ID NO: 89 - DNA, 91 bp, Artificial Sequence
  ssDNA2-2
ataccaatggcagagaccggtggcctgtatgcgtgccatatggggccaatgacctgggtgtgtcagccgttacgcggcgcagctcccgcag

SEQ ID NO: 90 - DNA, 156 bp, Artificial Sequence
  ssDNA2-3
ggcgcagctcccgcagcaccagctccagcagcaggcggtcgtatcgctcgtctggaagaaaaagttaaaaccctgaaagctcagaactccgaactggcttccaccgctaacatgctgcgtgaacaggttgctcagctgaaacagaaagttatgaac